European Patent Application EP 4 729 613 A1, published April 22, 2026. Title: ZINC FINGER NUCLEASE, VECTOR, AND METHODS FOR GENOME EDITTING AND PHOTORECEPTOR CELL PRODUCTION USING THERE OF. Applicant: VC GENE THERAPY. Application WO. The sequence listing filed with the application follows.

SEQUENCE LISTING (109 sequences)

SEQ ID NO: 1 - DNA, 18 bp, Homo sapiens
  source 1..18: mol_type = genomic DNA
attcttgggtgggagcag

SEQ ID NO: 2 - DNA, 18 bp, Homo sapiens
  source 1..18: mol_type = genomic DNA
aaggcctgagctcagcca

SEQ ID NO: 3 - DNA, 18 bp, Homo sapiens
  source 1..18: mol_type = genomic DNA
cttgggtgggagcagcca

SEQ ID NO: 4 - DNA, 18 bp, Homo sapiens
  source 1..18: mol_type = genomic DNA
gcgaaggcctgagctcag

SEQ ID NO: 5 - DNA, 18 bp, Homo sapiens
  source 1..18: mol_type = genomic DNA
gggtgggagcagccacgg

SEQ ID NO: 6 - DNA, 18 bp, Homo sapiens
  source 1..18: mol_type = genomic DNA
gctgcgaaggcctgagct

SEQ ID NO: 7 - DNA, 18 bp, Homo sapiens
  source 1..18: mol_type = genomic DNA
gtgggagcagccacgggt

SEQ ID NO: 8 - DNA, 18 bp, Homo sp.
  source 1..18: mol_type = genomic DNA
atgctgcgaaggcctgag

SEQ ID NO: 9 - DNA, 18 bp, Homo sapiens
  source 1..18: mol_type = genomic DNA
tgggagcagccacgggtc

SEQ ID NO: 10 - DNA, 18 bp, Homo sapiens
  source 1..18: mol_type = genomic DNA
aatgctgcgaaggcctga

SEQ ID NO: 11 - DNA, 18 bp, Homo sapiens
  source 1..18: mol_type = genomic DNA
ggagcagccacgggtcag

SEQ ID NO: 12 - DNA, 18 bp, Homo sapiens
  source 1..18: mol_type = genomic DNA
agaatgctgcgcaggcct

SEQ ID NO: 13 - DNA, 18 bp, Homo sapiens
  source 1..18: mol_type = genomic DNA
gagcagccacgggtcagc

SEQ ID NO: 14 - DNA, 18 bp, Homo sapiens
  source 1..18: mol_type = genomic DNA
aagaatgctgcgaaggcc

SEQ ID NO: 15 - DNA, 18 bp, Homo sapiens
  source 1..18: mol_type = genomic DNA
gcagccacgggtcagcca

SEQ ID NO: 16 - DNA, 18 bp, Homo sapiens
  source 1..18: mol_type = genomic DNA
ccaagaatgctgcgaagg

SEQ ID NO: 17 - DNA, 18 bp, Homo sapiens
  source 1..18: mol_type = genomic DNA
cagccacgggtcagccac

SEQ ID NO: 18 - DNA, 18 bp, Homo sapiens
  source 1..18: mol_type = genomic DNA
cccaagaatgctgcgaag

SEQ ID NO: 19 - DNA, 18 bp, Homo sapiens
  source 1..18: mol_type = genomic DNA
gccacgggtcagccacaa

SEQ ID NO: 20 - DNA, 18 bp, Homo sapiens
  source 1..18: mol_type = genomic DNA
cacccaagaatgctgcga

SEQ ID NO: 21 - DNA, 18 bp, Homo sapiens
  source 1..18: mol_type = genomic DNA
ccacgggtcagccacaag

SEQ ID NO: 22 - DNA, 18 bp, Homo sapiens
  source 1..18: mol_type = genomic DNA
ccacccaagaatgctgcg

SEQ ID NO: 23 - DNA, 18 bp, Homo sapiens
  source 1..18: mol_type = genomic DNA
gccacaagggccacagcc

SEQ ID NO: 24 - DNA, 18 bp, Homo sapiens
  source 1..18: mol_type = genomic DNA
gtggctgctcccacccaa

SEQ ID NO: 25 - DNA, 18 bp, Homo sapiens
  source 1..18: mol_type = genomic DNA
acaagggccacagccatg

SEQ ID NO: 26 - DNA, 18 bp, Homo sapiens
  source 1..18: mol_type = genomic DNA
cccgtggctgctcccacc

SEQ ID NO: 27 - DNA, 18 bp, Homo sapiens
  source 1..18: mol_type = genomic DNA
agggccacagccatgaat

SEQ ID NO: 28 - DNA, 18 bp, Homo sapiens
  source 1..18: mol_type = genomic DNA
tgacccgtggctgctccc

SEQ ID NO: 29 - DNA, 18 bp, Homo sapiens
  source 1..18: mol_type = genomic DNA
gccacagccatgaatggc

SEQ ID NO: 30 - DNA, 18 bp, Homo sapiens
  source 1..18: mol_type = genomic DNA
ggctgacccgtggctgct

SEQ ID NO: 31 - DNA, 18 bp, Homo sapiens
  source 1..18: mol_type = genomic DNA
cacagccatgaatggcac

SEQ ID NO: 32 - DNA, 18 bp, Homo sapiens
  source 1..18: mol_type = genomic DNA
gtggctgacccgtggctg

SEQ ID NO: 33 - DNA, 18 bp, Homo sapiens
  source 1..18: mol_type = genomic DNA
agccatgaatggcacaga

SEQ ID NO: 34 - DNA, 18 bp, Homo sapiens
  source 1..18: mol_type = genomic DNA
cttgtggctgacccgtgg

SEQ ID NO: 35 - DNA, 18 bp, Homo sapiens
  source 1..18: mol_type = genomic DNA
catgaatggcacagaagg

SEQ ID NO: 36 - DNA, 18 bp, Homo sapiens
  source 1..18: mol_type = genomic DNA
gcccttgtggctgacccg

SEQ ID NO: 37 - DNA, 18 bp, Homo sapiens
  source 1..18: mol_type = genomic DNA
tgggtgggagcagccacg

SEQ ID NO: 38 - DNA, 18 bp, Homo sapiens
  source 1..18: mol_type = genomic DNA
ggtgggagcagccacggg

SEQ ID NO: 39 - DNA, 18 bp, Homo sapiens
  source 1..18: mol_type = genomic DNA
gtcagccacaagggccac

SEQ ID NO: 40 - DNA, 18 bp, Homo sapiens
  source 1..18: mol_type = genomic DNA
gctgctcccacccaagaa

SEQ ID NO: 41 - DNA, 18 bp, Homo sapiens
  source 1..18: mol_type = genomic DNA
agccacaagggccacagc

SEQ ID NO: 42 - DNA, 18 bp, Homo sapiens
  source 1..18: mol_type = genomic DNA
cacaagggccacagccat

SEQ ID NO: 43 - DNA, 18 bp, Homo sapiens
  source 1..18: mol_type = genomic DNA
aagggccacagccatgaa

SEQ ID NO: 44 - DNA, 18 bp, Homo sapiens
  source 1..18: mol_type = genomic DNA
ggccacagccatgaatgg

SEQ ID NO: 45 - DNA, 18 bp, Homo sapiens
  source 1..18: mol_type = genomic DNA
ccacagccatgaatggca

SEQ ID NO: 46 - DNA, 18 bp, Homo sapiens
  source 1..18: mol_type = genomic DNA
cagccatgaatggcacag

SEQ ID NO: 47 - DNA, 18 bp, Homo sapiens
  source 1..18: mol_type = genomic DNA
ccatgaatggcacagaag

SEQ ID NO: 48 - DNA, 18 bp, Homo sapiens
  source 1..18: mol_type = genomic DNA
tgaatggcacagaaggcc

SEQ ID NO: 49 - DNA, 18 bp, Homo sapiens
  source 1..18: mol_type = genomic DNA
gtggcccttgtggctgac

SEQ ID NO: 50 - DNA, 18 bp, Homo sapiens
  source 1..18: mol_type = genomic DNA
atggcacagaaggcccta

SEQ ID NO: 51 - DNA, 18 bp, Homo sapiens
  source 1..18: mol_type = genomic DNA
gctgtggcccttgtggct

SEQ ID NO: 52 - protein, 585 aa, Bacillus sp. SGD-V-76
MATKRVVRTFGWIQNPGKFENLKRTVQVFDENSKVYKEVRDIKIPNLVKDKDVRTTLIAAMNRLENYYSYKELVGTGTSVRAQAPCDAIIQAAIQDQGNKKGYIDNWSSDGFVRWAHALGFLEYNSDKDSFYLTDIGLEYSRSTDDSLNEKIILIEALSSYPPAIRILTLLENGEHLTKFDLGKQLGFSGESGFTSLPQNLFLDALANAPSSPPTIKNSIRSDWEGSADKYARMISGWLVKMGLVAQGRKNFVVPTVGGSTRNEYISHAFKITKDGLDVLRRAKGASKHVRVPKRVYWEMFATNINDRVYVRTRRAYTLYLLMRSNTALNTVQLQVKLKALGFEELEETIENDVKGLINSGIFINVTNKGYHFKDTIKPFEIPEFGVTEPLVKGEMEKKKSDLRHKLKHVPHEYIELIEIAQDSKQNRLFEFKVVEFLKEVYDYNGKHLGGSRKPDGALYTNGLKTDYGIILDTKAYKDGYSLPISQADEMQRYVDENNNRNAIINPNEWWKVYPNSILDFKFLFVSGFFKGDYKKQLARVSNLTKRKGAVLSVEQLLLGGEKIKDGSLTLEDVGDKFNNDEIIF

SEQ ID NO: 53 - DNA, 1758 bp, Bacillus sp. SGD-V-76
  source 1..1758: mol_type = other DNA
atggcaacaaaacgagtggttcgtacatttggttggatacagaatccaggtaaattcgagaacctaaaacgaacagtccaagtattcgatgaaaactcaaaagtatataaagaggttagggatataaagattccaaatctagtgaaagataaagatgtaagaactactttaatagctgctatgaatcgattagaaaattattactcatataaagagttggttggtacaggtacttcagttagagctcaagcgccttgtgatgccattattcaagcagcgattcaagaccaaggtaataaaaaaggatacattgataattggtcttctgatggattcgttcgttgggcacatgcattggggtttcttgagtataactcagataaggactcattttacctaactgatattggattggaatattctcgttctacagatgattcactaaatgaaaaaatcatacttattgaagcattgtcatcatatccaccagcaattcgaatattgacattacttgaaaatggtgagcatttaacaaaattcgacctaggtaaacagttaggctttagtggagagagtggttttacttcattaccacaaaacttatttttagatgcgttagcaaatgcaccttcatcaccaccaacaattaagaattctattcgttctgattgggaaggttctgcggataaatatgcacggatgatttcaggctggcttgtaaagatggggcttgttgcacaaggtcgtaaaaattttgttgtaccaacggtaggtggttctactcgaaatgagtatatatctcatgcttttaaaattacaaaagatggtcttgatgtgttaaggagagcaaaaggtgccagtaaacatgtacgagtaccaaagcgtgtatactgggagatgttcgctaccaacattaacgatagagtgtatgtaagaacaagacgggcttatacactttacttgttaatgagaagtaacactgctctaaatactgttcaacttcaagtgaaattaaaagctttgggctttgaagaattggaagaaacaattgagaatgatgtaaaaggtttaattaactctggaatttttatcaatgtgacgaataaaggttatcattttaaagatacaattaaaccattcgaaattcctgaatttggcgtaacagaaccattagtaaagggggaaatggagaagaagaaatccgatttgcgtcataagttaaaacacgtaccgcatgaatatattgaactaatagaaattgcacaggattcaaagcaaaatcgtttgttcgaatttaaagtagttgagtttttgaaagaagtttatgattataatggaaagcacctaggggggagtcgaaaaccagatggcgcactatataccaatggtttaaaaacagattatggaataattttagataccaaagcttacaaagatggttatagtttaccaatctcccaggcagatgaaatgcagcgttatgtcgatgaaaataataatagaaatgctattattaatcctaacgaatggtggaaagtgtatcctaattctatcttggactttaaattcttattcgtaagtggtttttttaaaggtgactataaaaaacaattagctcgtgtaagtaatcttacaaagcgtaaaggtgctgtcctaagcgtagagcaactattattgggaggggaaaaaattaaagatggtagtttaacattagaagatgttggtgacaaattcaataatgatgaaattattttctaa

SEQ ID NO: 54 - protein, 579 aa, Clostridium botulinum
VESLRLSDITIRTFGWIQNPSDFSKLKKIVQLFDHTSSIHVDLKENRIPRLVEKDDGRDRFIEILNRIPLKIKYIDLVGTSFKPRSSGRCNGIAQAMIEGQGKSFTDNWTADGFIRWAHALGFIQYDYLEDEFSITQAGFDFSRSINDSEGENEILIEAMLSYPPAVRVLDLLSLGEHLTKFDIGKNLGFNGESGFTSLPLNIMLQTLADNDLVSEKTKIRQDWEGSSDKYSRMIAGWLSKLGLVKKGKKYFDVNIGGIIHREYISHAYKITGEGLKQLRRAKGTTSARRIEKRVCWEMFATKNLDRTYIRTRRAYILKFLEVSSSLITIEQIKTKLLEKGYDETVETIKSDIKGLINIGLNIQETTRGYSLKDSINDFMIPVTDLNQIVKSSIEMSKANMRDNLQMLPHDYIELIEISQDPYQNRIFEMKVMDLFINEYGFSGSHLGGSRKPDGAMYAHGFGVIVDTKAYKDGYNLPISQADEMERYVRENIDRNEHVNSNRWWNIFPEDTNEYKFLFVSGFFKGNFEKQLERISIDTGVQGGALSVEHLLLGAEYIKRGILTLYDFKNSFLNKEIQF

SEQ ID NO: 55 - DNA, 1740 bp, Clostridium botulinum
  source 1..1740: mol_type = other DNA
gtggaatcattaagattatcagacataacaattagaacatttgggtggattcagaatcctagtgattttagtaaattaaaaaaaatagttcagttatttgatcatacatcatctattcatgtggatttgaaagaaaaccgcataccacggttagtggagaaagatgacggacgtgataggtttattgagatattaaatcggattccgttaaagataaagtatattgatttagtaggaacatcatttaaacctagaagtagtggtagatgtaatggaattgctcaagcaatgattgaaggtcaaggtaagagttttactgataattggacagctgatgggtttattaggtgggctcatgcacttggctttatacaatatgattatttagaagatgagttttcaataacacaagcaggctttgatttttcaaggtcaatcaatgatagtgaaggggaaaatgaaatattaatagaggcaatgttgtcttatccacctgcagttagagttttagatttactttctttaggagagcatcttacaaaatttgatattggaaaaaatctgggcttcaatggcgaatcaggatttacatctttacctttaaatatcatgcttcaaacattagcagacaatgatttagtaagtgaaaagactaaaattcgtcaggattgggaaggttcttctgataagtattcacgaatgatagccggctggttatcgaaacttggtttggttaaaaagggaaaaaagtattttgatgtaaatattggaggaataattcatagagaatatatctctcatgcatataaaattactggagaaggtttaaaacaactccgtagggctaaaggaactacaagtgcaaggcgtatagaaaaacgggtttgctgggaaatgttcgccacaaagaatctagataggacatatattcgtacaagaagagcttatattttaaagtttttagaagtttcaagcagcttaattactattgagcaaattaagactaagttattggaaaaaggttatgacgaaacagtagaaactattaaatctgatattaaggggttaattaacattggtttaaatattcaagaaaccactcgaggttattcattaaaggattcaattaatgactttatgattccagtaaccgacttaaatcaaattgttaaaagtagtatagagatgtctaaagctaacatgagagacaatcttcagatgttgcctcatgattatattgagctaattgaaatatcacaagatccatatcaaaatagaatatttgaaatgaaagttatggatttatttattaatgagtatggtttcagtggttcgcacttaggtggaagtaggaaacctgatggtgctatgtatgcacatggttttggtgttattgttgatacaaaagcatataaagatgggtacaatcttcctataagtcaagctgatgaaatggaacgatatgtaagggaaaatattgatagaaatgaacatgtgaactcaaatagatggtggaatatatttcccgaagatacaaatgaatataagtttttattcgtaagtggtttctttaaaggaaattttgagaaacaattagaaaggataagtatagatactggtgtacaaggaggggctttaagtgttgaacatttattattaggtgctgagtacataaagaggggtattcttactttatatgattttaagaatagctttttaaataaggaaattcaattttaa

SEQ ID NO: 56 - protein, 4 aa, synthetic construct
TGGS

SEQ ID NO: 57 - protein, 195 aa, synthetic construct
LVKGEMEKKKSDLRHKLKHVPHEYIELIEIAQDSKQNRLFEFKVVEFLKEVYDYNGKHLGGSRKPDGALYTNGLKTDYGIILDTKAYKDGYSLPISQADEMQDYVDENNNRDAIINPNEWWKVYPNSILDFKFLFVSGFFKGDYKKQLARVSNLTKRKGAVLSVEQLLLGGEKIKDGSLTLEDVGDKFNNDEIIF

SEQ ID NO: 58 - protein, 195 aa, synthetic construct
LVKGEMEKKKSDLRHKLKHVPHEYIELIEIAQDSKQNRLFEFKVVEFLKEVYDYNGKHLGGSRKPDGALYTNGLKTDYGIILDTKAYKDGYSLPISQAREMQRYVDENNNRNAIINPNEWWKVYPNSILDFKFLFVSGFFKGDYKKQLARVSRLTKRKGAVLSVEQLLLGGEKIKDGSLTLEDVGDKFNNDEIIF

SEQ ID NO: 59 - protein, 168 aa, synthetic construct
PGEKPYKCPECGKSFSRADNLTEHQRTHTGEKPYKCPECGKSFSRSDNLVRHQRTHTGEKPYKCPECGKSFSRSDHLTTHQRTHTGEKPYKCPECGKSFSRSDKLVRHQRTHTGEKPYKCPECGKSFSTTGALTEHQRTHTGEKPYKCPECGKSFSHKNALQNHQRTH

SEQ ID NO: 60 - protein, 168 aa, synthetic construct
PGEKPYKCPECGKSFSTSHSLTEHQRTHTGEKPYKCPECGKSFSRADNLTEHQRTHTGEKPYKCPECGKSFSTSGELVRHQRTHTGEKPYKCPECGKSFSQAGHLASHQRTHTGEKPYKCPECGKSFSDCRDLARHQRTHTGEKPYKCPECGKSFSRKDNLKNHQRTH

SEQ ID NO: 61 - protein, 168 aa, synthetic construct
PGEKPYKCPECGKSFSTSHSLTEHQRTHTGEKPYKCPECGKSFSRADNLTEHQRTHTGEKPYKCPECGKSFSRSDNLVRHQRTHTGEKPYKCPECGKSFSRSDHLTTHQRTHTGEKPYKCPECGKSFSRSDKLVRHQRTHTGEKPYKCPECGKSFSTTGALTEHQRTH

SEQ ID NO: 62 - protein, 168 aa, synthetic construct
PGEKPYKCPECGKSFSRADNLTEHQRTHTGEKPYKCPECGKSFSTSGELVRHQRTHTGEKPYKCPECGKSFSQAGHLASHQRTHTGEKPYKCPECGKSFSDCRDLARHQRTHTGEKPYKCPECGKSFSRKDNLKNHQRTHTGEKPYKCPECGKSFSRSDDLVRHQRTH

SEQ ID NO: 63 - protein, 168 aa, synthetic construct
PGEKPYKCPECGKSFSRSDKLTEHQRTHTGEKPYKCPECGKSFSTSHSLTEHQRTHTGEKPYKCPECGKSFSRADNLTEHQRTHTGEKPYKCPECGKSFSRSDNLVRHQRTHTGEKPYKCPECGKSFSRSDHLTTHQRTHTGEKPYKCPECGKSFSRSDKLVRHQRTH

SEQ ID NO: 64 - protein, 168 aa, synthetic construct
PGEKPYKCPECGKSFSTSGELVRHQRTHTGEKPYKCPECGKSFSQAGHLASHQRTHTGEKPYKCPECGKSFSDCRDLARHQRTHTGEKPYKCPECGKSFSRKDNLKNHQRTHTGEKPYKCPECGKSFSRSDDLVRHQRTHTGEKPYKCPECGKSFSTSGELVRHQRTH

SEQ ID NO: 65 - protein, 168 aa, synthetic construct
PGEKPYKCPECGKSFSTSGHLVRHQRTHTGEKPYKCPECGKSFSRTDTLRDHQRTHTGEKPYKCPECGKSFSDCRDLARHQRTHTGEKPYKCPECGKSFSQSGDLRRHQRTHTGEKPYKCPECGKSFSQRAHLERHQRTHTGEKPYKCPECGKSFSRSDELVRHQRTH

SEQ ID NO: 66 - protein, 168 aa, synthetic construct
PGEKPYKCPECGKSFSRSDNLVRHQRTHTGEKPYKCPECGKSFSTKNSLTEHQRTHTGEKPYKCPECGKSFSRSDHLTNHQRTHTGEKPYKCPECGKSFSQSGHLTEHQRTHTGEKPYKCPECGKSFSRNDALTEHQRTHTGEKPYKCPECGKSFSRRDELNVHQRTH

SEQ ID NO: 67 - protein, 168 aa, synthetic construct
PGEKPYKCPECGKSFSDPGALVRHQRTHTGEKPYKCPECGKSFSRSDKLTEHQRTHTGEKPYKCPECGKSFSTSHSLTEHQRTHTGEKPYKCPECGKSFSRADNLTEHQRTHTGEKPYKCPECGKSFSRSDNLVRHQRTHTGEKPYKCPECGKSFSRSDHLTTHQRTH

SEQ ID NO: 68 - protein, 168 aa, synthetic construct
PGEKPYKCPECGKSFSQAGHLASHQRTHTGEKPYKCPECGKSFSDCRDLARHQRTHTGEKPYKCPECGKSFSRKDNLKNHQRTHTGEKPYKCPECGKSFSRSDDLVRHQRTHTGEKPYKCPECGKSFSTSGELVRHQRTHTGEKPYKCPECGKSFSTTGNLTVHQRTH

SEQ ID NO: 69 - protein, 168 aa, synthetic construct
PGEKPYKCPECGKSFSRADNLTEHQRTHTGEKPYKCPECGKSFSTSGHLVRHQRTHTGEKPYKCPECGKSFSRTDTLRDHQRTHTGEKPYKCPECGKSFSDCRDLARHQRTHTGEKPYKCPECGKSFSQSGDLRRHQRTHTGEKPYKCPECGKSFSQRAHLERHQRTH

SEQ ID NO: 70 - protein, 168 aa, synthetic construct
PGEKPYKCPECGKSFSTKNSLTEHQRTHTGEKPYKCPECGKSFSRSDHLTNHQRTHTGEKPYKCPECGKSFSQSGHLTEHQRTHTGEKPYKCPECGKSFSRNDALTEHQRTHTGEKPYKCPECGKSFSRRDELNVHQRTHTGEKPYKCPECGKSFSQLAHLRAHQRTH

SEQ ID NO: 71 - protein, 168 aa, synthetic construct
PGEKPYKCPECGKSFSERSHLREHQRTHTGEKPYKCPECGKSFSDPGALVRHQRTHTGEKPYKCPECGKSFSRSDKLTEHQRTHTGEKPYKCPECGKSFSTSHSLTEHQRTHTGEKPYKCPECGKSFSRADNLTEHQRTHTGEKPYKCPECGKSFSRSDNLVRHQRTH

SEQ ID NO: 72 - protein, 168 aa, synthetic construct
PGEKPYKCPECGKSFSDCRDLARHQRTHTGEKPYKCPECGKSFSRKDNLKNHQRTHTGEKPYKCPECGKSFSRSDDLVRHQRTHTGEKPYKCPECGKSFSTSGELVRHQRTHTGEKPYKCPECGKSFSTTGNLTVHQRTHTGEKPYKCPECGKSFSRKDNLKNHQRTH

SEQ ID NO: 73 - protein, 168 aa, synthetic construct
PGEKPYKCPECGKSFSTSHSLTEHQRTHTGEKPYKCPECGKSFSRADNLTEHQRTHTGEKPYKCPECGKSFSTSGHLVRHQRTHTGEKPYKCPECGKSFSRTDTLRDHQRTHTGEKPYKCPECGKSFSDCRDLARHQRTHTGEKPYKCPECGKSFSQSGDLRRHQRTH

SEQ ID NO: 74 - protein, 168 aa, synthetic construct
PGEKPYKCPECGKSFSRSDHLTNHQRTHTGEKPYKCPECGKSFSQSGHLTEHQRTHTGEKPYKCPECGKSFSRNDALTEHQRTHTGEKPYKCPECGKSFSRRDELNVHQRTHTGEKPYKCPECGKSFSQLAHLRAHQRTHTGEKPYKCPECGKSFSTSHSLTEHQRTH

SEQ ID NO: 75 - protein, 168 aa, synthetic construct
PGEKPYKCPECGKSFSSKKALTEHQRTHTGEKPYKCPECGKSFSERSHLREHQRTHTGEKPYKCPECGKSFSDPGALVRHQRTHTGEKPYKCPECGKSFSRSDKLTEHQRTHTGEKPYKCPECGKSFSTSHSLTEHQRTHTGEKPYKCPECGKSFSRADNLTEHQRTH

SEQ ID NO: 76 - protein, 168 aa, synthetic construct
PGEKPYKCPECGKSFSRKDNLKNHQRTHTGEKPYKCPECGKSFSRSDDLVRHQRTHTGEKPYKCPECGKSFSTSGELVRHQRTHTGEKPYKCPECGKSFSTTGNLTVHQRTHTGEKPYKCPECGKSFSRKDNLKNHQRTHTGEKPYKCPECGKSFSSKKHLAEHQRTH

SEQ ID NO: 77 - protein, 168 aa, synthetic construct
PGEKPYKCPECGKSFSQSGNLTEHQRTHTGEKPYKCPECGKSFSTSHSLTEHQRTHTGEKPYKCPECGKSFSRADNLTEHQRTHTGEKPYKCPECGKSFSTSGHLVRHQRTHTGEKPYKCPECGKSFSRTDTLRDHQRTHTGEKPYKCPECGKSFSDCRDLARHQRTH

SEQ ID NO: 78 - protein, 168 aa, synthetic construct
PGEKPYKCPECGKSFSQSGHLTEHQRTHTGEKPYKCPECGKSFSRNDALTEHQRTHTGEKPYKCPECGKSFSRRDELNVHQRTHTGEKPYKCPECGKSFSQLAHLRAHQRTHTGEKPYKCPECGKSFSTSHSLTEHQRTHTGEKPYKCPECGKSFSSKKALTEHQRTH

SEQ ID NO: 79 - protein, 168 aa, synthetic construct
PGEKPYKCPECGKSFSRKDNLKNHQRTHTGEKPYKCPECGKSFSSKKALTEHQRTHTGEKPYKCPECGKSFSERSHLREHQRTHTGEKPYKCPECGKSFSDPGALVRHQRTHTGEKPYKCPECGKSFSRSDKLTEHQRTHTGEKPYKCPECGKSFSTSHSLTEHQRTH

SEQ ID NO: 80 - protein, 168 aa, synthetic construct
PGEKPYKCPECGKSFSRSDDLVRHQRTHTGEKPYKCPECGKSFSTSGELVRHQRTHTGEKPYKCPECGKSFSTTGNLTVHQRTHTGEKPYKCPECGKSFSRKDNLKNHQRTHTGEKPYKCPECGKSFSSKKHLAEHQRTHTGEKPYKCPECGKSFSTSHSLTEHQRTH

SEQ ID NO: 81 - protein, 168 aa, synthetic construct
PGEKPYKCPECGKSFSDCRDLARHQRTHTGEKPYKCPECGKSFSSPADLTRHQRTHTGEKPYKCPECGKSFSDCRDLARHQRTHTGEKPYKCPECGKSFSRSDHLTNHQRTHTGEKPYKCPECGKSFSSPADLTRHQRTHTGEKPYKCPECGKSFSDCRDLARHQRTH

SEQ ID NO: 82 - protein, 168 aa, synthetic construct
PGEKPYKCPECGKSFSQSGNLTEHQRTHTGEKPYKCPECGKSFSDKKDLTRHQRTHTGEKPYKCPECGKSFSSKKHLAEHQRTHTGEKPYKCPECGKSFSTSGELVRHQRTHTGEKPYKCPECGKSFSTSGELVRHQRTHTGEKPYKCPECGKSFSRSDELVRHQRTH

SEQ ID NO: 83 - protein, 168 aa, synthetic construct
PGEKPYKCPECGKSFSRRDELNVHQRTHTGEKPYKCPECGKSFSDCRDLARHQRTHTGEKPYKCPECGKSFSSPADLTRHQRTHTGEKPYKCPECGKSFSDCRDLARHQRTHTGEKPYKCPECGKSFSRSDHLTNHQRTHTGEKPYKCPECGKSFSSPADLTRHQRTH

SEQ ID NO: 84 - protein, 168 aa, synthetic construct
PGEKPYKCPECGKSFSDKKDLTRHQRTHTGEKPYKCPECGKSFSSKKHLAEHQRTHTGEKPYKCPECGKSFSTSGELVRHQRTHTGEKPYKCPECGKSFSTSGELVRHQRTHTGEKPYKCPECGKSFSRSDELVRHQRTHTGEKPYKCPECGKSFSSKKHLAEHQRTH

SEQ ID NO: 85 - protein, 168 aa, synthetic construct
PGEKPYKCPECGKSFSTTGNLTVHQRTHTGEKPYKCPECGKSFSRRDELNVHQRTHTGEKPYKCPECGKSFSDCRDLARHQRTHTGEKPYKCPECGKSFSSPADLTRHQRTHTGEKPYKCPECGKSFSDCRDLARHQRTHTGEKPYKCPECGKSFSRSDHLTNHQRTH

SEQ ID NO: 86 - protein, 168 aa, synthetic construct
PGEKPYKCPECGKSFSSKKHLAEHQRTHTGEKPYKCPECGKSFSTSGELVRHQRTHTGEKPYKCPECGKSFSTSGELVRHQRTHTGEKPYKCPECGKSFSRSDELVRHQRTHTGEKPYKCPECGKSFSSKKHLAEHQRTHTGEKPYKCPECGKSFSQAGHLASHQRTH

SEQ ID NO: 87 - protein, 168 aa, synthetic construct
PGEKPYKCPECGKSFSDPGHLVRHQRTHTGEKPYKCPECGKSFSTTGNLTVHQRTHTGEKPYKCPECGKSFSRRDELNVHQRTHTGEKPYKCPECGKSFSDCRDLARHQRTHTGEKPYKCPECGKSFSSPADLTRHQRTHTGEKPYKCPECGKSFSDCRDLARHQRTH

SEQ ID NO: 88 - protein, 168 aa, synthetic construct
PGEKPYKCPECGKSFSTSGELVRHQRTHTGEKPYKCPECGKSFSTSGELVRHQRTHTGEKPYKCPECGKSFSRSDELVRHQRTHTGEKPYKCPECGKSFSSKKHLAEHQRTHTGEKPYKCPECGKSFSQAGHLASHQRTHTGEKPYKCPECGKSFSDPGHLVRHQRTH

SEQ ID NO: 89 - protein, 168 aa, synthetic construct
PGEKPYKCPECGKSFSSKKALTEHQRTHTGEKPYKCPECGKSFSRSDHLTTHQRTHTGEKPYKCPECGKSFSQSSNLVRHQRTHTGEKPYKCPECGKSFSTSGNLTEHQRTHTGEKPYKCPECGKSFSERSHLREHQRTHTGEKPYKCPECGKSFSSKKALTEHQRTH

SEQ ID NO: 90 - protein, 168 aa, synthetic construct
PGEKPYKCPECGKSFSRNDALTEHQRTHTGEKPYKCPECGKSFSRSDHLTTHQRTHTGEKPYKCPECGKSFSRNDTLTEHQRTHTGEKPYKCPECGKSFSDPGNLVRHQRTHTGEKPYKCPECGKSFSTSGELVRHQRTHTGEKPYKCPECGKSFSRSDELVRHQRTH

SEQ ID NO: 91 - protein, 168 aa, synthetic construct
PGEKPYKCPECGKSFSQLAHLRAHQRTHTGEKPYKCPECGKSFSSKKALTEHQRTHTGEKPYKCPECGKSFSRSDHLTTHQRTHTGEKPYKCPECGKSFSQSSNLVRHQRTHTGEKPYKCPECGKSFSTSGNLTEHQRTHTGEKPYKCPECGKSFSERSHLREHQRTH

SEQ ID NO: 92 - protein, 168 aa, synthetic construct
PGEKPYKCPECGKSFSRSDHLTTHQRTHTGEKPYKCPECGKSFSRNDTLTEHQRTHTGEKPYKCPECGKSFSDPGNLVRHQRTHTGEKPYKCPECGKSFSTSGELVRHQRTHTGEKPYKCPECGKSFSRSDELVRHQRTHTGEKPYKCPECGKSFSTTGALTEHQRTH

SEQ ID NO: 93 - protein, 168 aa, synthetic construct
PGEKPYKCPECGKSFSRSDHLTNHQRTHTGEKPYKCPECGKSFSQLAHLRAHQRTHTGEKPYKCPECGKSFSSKKALTEHQRTHTGEKPYKCPECGKSFSRSDHLTTHQRTHTGEKPYKCPECGKSFSQSSNLVRHQRTHTGEKPYKCPECGKSFSTSGNLTEHQRTH

SEQ ID NO: 94 - protein, 168 aa, synthetic construct
PGEKPYKCPECGKSFSRNDTLTEHQRTHTGEKPYKCPECGKSFSDPGNLVRHQRTHTGEKPYKCPECGKSFSTSGELVRHQRTHTGEKPYKCPECGKSFSRSDELVRHQRTHTGEKPYKCPECGKSFSTTGALTEHQRTHTGEKPYKCPECGKSFSDCRDLARHQRTH

SEQ ID NO: 95 - protein, 168 aa, synthetic construct
PGEKPYKCPECGKSFSRTDTLRDHQRTHTGEKPYKCPECGKSFSDCRDLARHQRTHTGEKPYKCPECGKSFSQSGDLRRHQRTHTGEKPYKCPECGKSFSQRAHLERHQRTHTGEKPYKCPECGKSFSRSDELVRHQRTHTGEKPYKCPECGKSFSRSDHLTTHQRTH

SEQ ID NO: 96 - protein, 168 aa, synthetic construct
PGEKPYKCPECGKSFSRSDKLVRHQRTHTGEKPYKCPECGKSFSSKKALTEHQRTHTGEKPYKCPECGKSFSERSHLREHQRTHTGEKPYKCPECGKSFSERSHLREHQRTHTGEKPYKCPECGKSFSRSDKLVRHQRTHTGEKPYKCPECGKSFSTSGHLVRHQRTH

SEQ ID NO: 97 - protein, 168 aa, synthetic construct
PGEKPYKCPECGKSFSSKKALTEHQRTHTGEKPYKCPECGKSFSDPGHLVRHQRTHTGEKPYKCPECGKSFSRKDNLKNHQRTHTGEKPYKCPECGKSFSSKKALTEHQRTHTGEKPYKCPECGKSFSERSHLREHQRTHTGEKPYKCPECGKSFSDPGALVRHQRTH

SEQ ID NO: 98 - protein, 168 aa, synthetic construct
PGEKPYKCPECGKSFSQSSNLVRHQRTHTGEKPYKCPECGKSFSQSGNLTEHQRTHTGEKPYKCPECGKSFSDKKDLTRHQRTHTGEKPYKCPECGKSFSSKKHLAEHQRTHTGEKPYKCPECGKSFSTSGELVRHQRTHTGEKPYKCPECGKSFSTSGELVRHQRTH

SEQ ID NO: 99 - protein, 168 aa, synthetic construct
PGEKPYKCPECGKSFSERSHLREHQRTHTGEKPYKCPECGKSFSSKKALTEHQRTHTGEKPYKCPECGKSFSDPGHLVRHQRTHTGEKPYKCPECGKSFSRKDNLKNHQRTHTGEKPYKCPECGKSFSSKKALTEHQRTHTGEKPYKCPECGKSFSERSHLREHQRTH

SEQ ID NO: 100 - protein, 168 aa, synthetic construct; identical to SEQ ID NO: 84

SEQ ID NO: 101 - protein, 168 aa, synthetic construct
PGEKPYKCPECGKSFSQSSNLVRHQRTHTGEKPYKCPECGKSFSTSGNLTEHQRTHTGEKPYKCPECGKSFSERSHLREHQRTHTGEKPYKCPECGKSFSSKKALTEHQRTHTGEKPYKCPECGKSFSDPGHLVRHQRTHTGEKPYKCPECGKSFSRKDNLKNHQRTH

SEQ ID NO: 102 - protein, 168 aa, synthetic construct
PGEKPYKCPECGKSFSRSDHLTTHQRTHTGEKPYKCPECGKSFSQSSNLVRHQRTHTGEKPYKCPECGKSFSTSGNLTEHQRTHTGEKPYKCPECGKSFSERSHLREHQRTHTGEKPYKCPECGKSFSSKKALTEHQRTHTGEKPYKCPECGKSFSDPGHLVRHQRTH

SEQ ID NO: 103 - protein, 168 aa, synthetic construct
PGEKPYKCPECGKSFSQSGDLRRHQRTHTGEKPYKCPECGKSFSRRDELNVHQRTHTGEKPYKCPECGKSFSQAGHLASHQRTHTGEKPYKCPECGKSFSTSHSLTEHQRTHTGEKPYKCPECGKSFSRADNLTEHQRTHTGEKPYKCPECGKSFSTSHSLTEHQRTH

SEQ ID NO: 104 - protein, 168 aa, synthetic construct
PGEKPYKCPECGKSFSRADNLTEHQRTHTGEKPYKCPECGKSFSQSGDLRRHQRTHTGEKPYKCPECGKSFSRRDELNVHQRTHTGEKPYKCPECGKSFSQAGHLASHQRTHTGEKPYKCPECGKSFSTSHSLTEHQRTHTGEKPYKCPECGKSFSRADNLTEHQRTH

SEQ ID NO: 105 - protein, 168 aa, synthetic construct
PGEKPYKCPECGKSFSRKDNLKNHQRTHTGEKPYKCPECGKSFSRADNLTEHQRTHTGEKPYKCPECGKSFSQSGDLRRHQRTHTGEKPYKCPECGKSFSRRDELNVHQRTHTGEKPYKCPECGKSFSQAGHLASHQRTHTGEKPYKCPECGKSFSTSHSLTEHQRTH

SEQ ID NO: 106 - protein, 168 aa, synthetic construct
PGEKPYKCPECGKSFSDCRDLARHQRTHTGEKPYKCPECGKSFSRKDNLKNHQRTHTGEKPYKCPECGKSFSRADNLTEHQRTHTGEKPYKCPECGKSFSQSGDLRRHQRTHTGEKPYKCPECGKSFSRRDELNVHQRTHTGEKPYKCPECGKSFSQAGHLASHQRTH

SEQ ID NO: 107 - protein, 168 aa, synthetic construct
PGEKPYKCPECGKSFSDPGNLVRHQRTHTGEKPYKCPECGKSFSTSGELVRHQRTHTGEKPYKCPECGKSFSRSDELVRHQRTHTGEKPYKCPECGKSFSTTGALTEHQRTHTGEKPYKCPECGKSFSDCRDLARHQRTHTGEKPYKCPECGKSFSRSDELVRHQRTH

SEQ ID NO: 108 - protein, 168 aa, synthetic construct
PGEKPYKCPECGKSFSQNSTLTEHQRTHTGEKPYKCPECGKSFSDCRDLARHQRTHTGEKPYKCPECGKSFSRKDNLKNHQRTHTGEKPYKCPECGKSFSRADNLTEHQRTHTGEKPYKCPECGKSFSQSGDLRRHQRTHTGEKPYKCPECGKSFSRRDELNVHQRTH

SEQ ID NO: 109 - protein, 168 aa, synthetic construct
PGEKPYKCPECGKSFSTSGELVRHQRTHTGEKPYKCPECGKSFSRSDELVRHQRTHTGEKPYKCPECGKSFSTTGALTEHQRTHTGEKPYKCPECGKSFSDCRDLARHQRTHTGEKPYKCPECGKSFSRSDELVRHQRTHTGEKPYKCPECGKSFSTSGELVRHQRTH